European Patent Application EP 4 715 050 A1, published March 25, 2026. Title: PET 분해 활성을 갖는 변이형 폴리펩티드. Applicant: 주식회사 자이엔. Application KR. The sequence listing filed with the application follows.

SEQUENCE LISTING (18 sequences)

SEQ ID NO: 1 - protein, 290 aa, Ideonella sakaensis
MNFPRASRLMQAAVLGGLMAVSAAATAQTNPYARGPNPTAASLEASAGPFTVRSFTVSRPSGYGAGTVYYPTNAGGTVGAIAIVPGYTARQSSIKWWGPRLASHGFVVITIDTNSTLDQPSSRSSQQMAALRQVASLNGTSSSPIYGKVDTARMGVMGWSMGGGGSLISAANNPSLKAAAPQAPWDSSTNFSSVTVPTLIFACENDSIAPVNSSALPIYDSMSRNAKQFLEINGGSHSCANSGNSNQALIGKKGVAWMKRFMDNDTRYSTFACENPNSTRVSDFRTANCS

SEQ ID NO: 2 - DNA, 873 bp, Ideonella sakaensis
  source 1..873: mol_type = genomic DNA
atgaactttccccgcgcttcccgcctgatgcaggccgccgttctcggcgggctgatggccgtgtcggccgccgccaccgcccagaccaacccctacgcccgcggcccgaacccgacagccgcctcactcgaagccagcgccggcccgttcaccgtgcgctcgttcaccgtgagccgcccgagcggctacggcgccggcaccgtgtactaccccaccaacgccggcggcaccgtgggcgccatcgccatcgtgccgggctacaccgcgcgccagtcgagcatcaaatggtggggcccgcgcctggcctcgcacggcttcgtggtcatcaccatcgacaccaactccacgctcgaccagccgtccagccgctcgtcgcagcagatggccgcgctgcgccaggtggcctcgctcaacggcaccagcagcagcccgatctacggcaaggtcgacaccgcccgcatgggcgtgatgggctggtcgatgggcggtggcggctcgctgatctcggcggccaacaacccgtcgctgaaagccgcggcgccgcaggccccgtgggacagctcgaccaacttctcgtcggtcaccgtgcccacgctgatcttcgcctgcgagaacgacagcatcgccccggtcaactcgtccgccctgccgatctacgacagcatgtcgcgcaatgcgaagcagttcctcgagatcaacggtggctcgcactcctgcgccaacagcggcaacagcaaccaggcgctgatcggcaagaagggcgtggcctggatgaagcgcttcatggacaacgacacgcgctactccaccttcgcctgcgagaacccgaacagcacccgcgtgtcggacttccgcaccgcgaactgcagctga

SEQ ID NO: 3 - protein, 290 aa, synthetic construct
  source 1..290: note = IsPETaseM1
MNFPRASRLMQAAVLGGLMAVSAAATAQTNPYARGPNPTAASLEASAGPFTVRSFTVSRPSGYGAGTVYYPTNAGGTVGAIAIVPGYTARQSSIKWWGPRLASHGFVVITIDTNSTLDQPSSRSSQQMAALRQVASLNGTSSSPIYGKVDTARMGVMGWSMGGGGSLISAANNPSLKAAAVQAPWDSSTNFSSVTVPTLIFACENDSIAPVNSSALPIYDSMSRNAKQFLEINGGSHSCANSGNSNQALIGKKGVAWMKRFMDNDTRYSTFACENPNSTRVSDFRTANCS

SEQ ID NO: 4 - protein, 290 aa, synthetic construct
  source 1..290: note = IsPETaseM2
MNFPRASRLMQAAVLGGLMAVSAAATAQTNPYARGPNPTAASLEASAGPFTVRSFTVSRPSGYGAGTVYYPTNAGGTVGAIAIVPGYTARQSSIKWWGPRLASHGFVVITIDTNSTLDQPSSRSSQQMAALRQVASLNGTSSSPIYGKVDTARMGVMGWSMGGGGSLISAANNPSLKAAVPQAPWDSSTNFSSVTVPTLIFACENDSIAPVNSSALPIYDSMSRNAKQFLEINGGSHSCANSGNSNQALIGKKGVAWMKRFMDNDTRYSTFACENPNSTRVSDFRTANCS

SEQ ID NO: 5 - protein, 290 aa, synthetic construct
  source 1..290: note = IsPETaseM3
MNFPRASRLMQAAVLGGLMAVSAAATAQTNPYARGPDPTAASLEASAGPFTVRSFTVSRPSGYGAGTVYYPTNAGGTVGAIAIVPGYTARQSSIKWWGPRLASHGFVVITIDTNSTLDQPSSRSSQQMAALRQVASLNGTSSSPIYGKVDTARMGVMGWSMGGGGSLISAANNPSLKAAAPQAPWDSSTNFSSVTVPTLIFACENDSIAPVNSSALPIYDSMSRNAKQFLEINGGSHSCANSGNSNQALIGKKGVAWMKRFMDNDTRYSTFACENPNSTRVSDFRTANCS

SEQ ID NO: 6 - protein, 290 aa, synthetic construct
  source 1..290: note = IsPETaseM4
MNFPRASRLMQAAVLGGLMAVSAAATAQTNPYARGPNPTAASLEASAGPFTVRSFTVSRPSGYGAGTVYYPTNAGGTVGAIAIVPGYTARQSSIKWWGPRLASHGFVVITIDTNSTLDQPSSRSSQQMAALEQVASLNGTSSSPIYGKVDTARMGVMGWSMGGGGSLISAANNPSLKAAAPQAPWDSSTNFSSVTVPTLIFACENDSIAPVNSSALPIYDSMSRNAKQFLEINGGSHSCANSGNSNQALIGKKGVAWMKRFMDNDTRYSTFACENPNSTRVSDFRTANCS

SEQ ID NO: 7 - protein, 290 aa, synthetic construct
  source 1..290: note = IsPETaseM5
MNFPRASRLMQAAVLGGLMAVSAAATAQTNPYARGPNPTAASLEASAGPFTVRSFTVSRPSGYGAGTVYYPTNAGGTVGAIAIVPGYTARQSSIKWWGPRLASHGFVVITIDTNSTLDQPSSRSSQQMAALRQVASLNGTSSSPIYGKVDTARMGVMGWSMGGGGSLISACNNPSLKAAAPQAPWDSSTNFSCVTVPTLIFACENDSIAPVNSSALPIYDSMSRNAKQFLEINGGSHSCANSGNSNQALIGKKGVAWMKRFMDNDTRYSTFACENPNSTRVSDFRTANCS

SEQ ID NO: 8 - protein, 290 aa, synthetic construct
  source 1..290: note = IsPETaseM6
MNFPRASRLMQAAVLGGLMAVSAAATAQTNPYARGPNPTAASLEASAGPFTVRSFTVSRPSGYGAGTVYYPTNAGGTVGAIAIVPGYTARQSSIKWWGPRLASHGFVVITIDTNSTLDQPSSRSSQQMAALRQVASLNGTSSSPIYGKVDTARMGVMGWSMGGGGSLISAANNPSLKAAAPQAPWDSSTNFSSVTVPTLIFCCENDSIAPCNSSALPIYDSMSRNAKQFLEINGGSHSCANSGNSNQALIGKKGVAWMKRFMDNDTRYSTFACENPNSTRVSDFRTANCS

SEQ ID NO: 9 - protein, 290 aa, synthetic construct
  source 1..290: note = IsPETaseM7
MNFPRASRLMQAAVLGGLMAVSAAATAQTNPYARGPNPTAASLEASAGPFTVRSFTVSRPSGYGAGTVYYPTNAGGTVGAIAIVPGYTARQSSIKWWGPRLASHGFVVITIDTNSTLDQPSSRSSQQMAALRQVASLNGTSSSPIYGKVDTARMGVMGWSMGGGGSLISAANNPSLKAAAPQAPWDSSTNFSSVTVPTLIFACENDSIAPVNSSALPIYDSMSRNAKQFLEINGGSHSCANSGNSNQALIGKKGVAWMKRFMDNDTRYSTFACECPNSTRVSDCRTANCS

SEQ ID NO: 10 - protein, 290 aa, synthetic construct
  source 1..290: note = IsPETaseM8
MNFPRASRLMQAAVLGGLMAVSAAATAQTNPYARGPNPTAASLEASAGPFTVRSFTVSRPSGYGAGTVYYPTNAGGTVGAIAIVPGYTARQSSIKWWGPRLASHGFVVITIDTNSTLDQPSSRSSQQMAALRQVASLNGTSSSPIYGKVDTARMGVMGWSMGGGGSLISAANNPSLKAAAPQAPWDSSTNFSSVTVPTLIFACENDSIAPVNSYALPIYDSMSRNAKQFLEINGGSHSCANSGNSNQALIGKKGVAWMKRFMDNDTRYSTFACENPNSTRVSDFRTANCS

SEQ ID NO: 11 - protein, 290 aa, synthetic construct
  source 1..290: note = IsPETaseM9
MNFPRASRLMQAAVLGGLMAVSAAATAQTNPYARGPNPTAASLEASAGPFTVRSFTVSDPSGYGAGTVYYPTNAGGTVGAIAIVPGYTARQSSIKWWGPRLASHGFVVITIDTNSTLDQPSSRSSQQMAALRQVASLNGTSSSPIYGKVDTARMGVMGWSMGGGGSLISAANNPSLKAAAPQAPWDSSTNFSSVTVPTLIFACENDSIAPVNSSALPIYDSMSRNAKQFLEINGGSHSCANSGNSNQALIGKKGVAWMKRFMDNDTRYSTFACENPNSTRVSDFRTANCS

SEQ ID NO: 12 - protein, 290 aa, synthetic construct
  source 1..290: note = IsPETaseM10
MNFPRASRLMQAAVLGGLMAVSAAATAQTNPYARGPNPTAASLEASAGPFTVRSFTVSRPSGYGAGTVYYPTNAGGTVGAIAIVPGYTARQSSIKWWGPRLASHGFVVITIDTNSTLDQPSSRSSQQMAALRQVASLNGTSSSPIYGKVDTARMGVMGWSMGGGGSLISAANNPSLKAAAPQAPWDSSTNFSSVTVPTLIFACENDSIAPVNSSALPIYDSMSHNAKQFLEINGGSHSCANSGNSNQALIGKKGVAWMKRFMDNDTRYSTFACENPNSTRVSDFRTANCS

SEQ ID NO: 13 - protein, 290 aa, synthetic construct
  source 1..290: note = IsPETaseM11
MNFPRASRLMQAAVLGGLMAVSAAATAQTNPYARGPNPTAASLEASAGPFTVRSFTVSRPSGYGAGTVYYPTNAGGTVGAIAIVPGYTARQSSIKWWGPRLASHGFVVITIDTNSTLDQPSSRSSQQMAALRQVASLNGTSSSPIYGKVDTARMGVMGWSMGGGGSLISAANNPSLKAAAPQAPWDSSTNFSSVTVPTLIFACENDSIAPVNSSALPIYDSMSRNAKQFLVINGGSHSCANSGNSNQALIGKKGVAWMKRFMDNDTRYSTFACENPNSTRVSDFRTANCS

SEQ ID NO: 14 - protein, 290 aa, synthetic construct
  source 1..290: note = IsPETaseM12
MNFPRASRLMQAAVLGGLMAVSAAATAQTNPYARGPNPTAASLEASAGPFTVRSFTVSRPSGYGAGTVYYPTNAGGTVGAIAIVPGYTARQSSIKWWGPRLASHGFVVITIDTNSTLDQPSSRSSQQMAALRQVASLNGTSSSPIYGKVDTARMGVMGWSMGGGGSLISAANNPSLKAAAPQAPWDSSTNFSSVTVPTLIFACENDSIAPVNSSALAIYDSMSRNAKQFLEINGGSHSCANSGNSNQALIGKKGVAWMKRFMDNDTRYSTFACENPNSTRVSDFRTANCS

SEQ ID NO: 15 - DNA, 30 bp, synthetic construct
  source 1..30: mol_type = other DNA; note = IsPETase variant F
gcgccatatgcgcggcccggatccgacagc

SEQ ID NO: 16 - DNA, 29 bp, synthetic construct
  source 1..29: mol_type = other DNA; note = IsPETase variant R
cgcgctcgagctgcaattcgctgtacgaa

SEQ ID NO: 17 - protein, 290 aa, synthetic construct
  source 1..290: note = IsPETaseM239
MNFPRASRLMQAAVLGGLMAVSAAATAQTNPYARGPDPTAASLEASAGPFTVRSFTVSRPSGYGAGTVYYPTNAGGTVGAIAIVPGYTARQSSIKWWGPRLASHGFVVITIDTNSTLDQPESRSSQQMAALEQVASLNGTSSSPIYGKVDTARMGVMGWSMGGGGSLISACNNPSLKAAVVQAPWHSSTNFSCVTVPTLIFACENDSIAPVNSSALPIYDSMSENAKQFLEICGGSHSCANTGNSDQALIGKKGVAWMKRFMDNDTRYSTFACENPNSTRVCDFRTANCS

SEQ ID NO: 18 - protein, 290 aa, synthetic construct
  source 1..290: note = IsPETaseM242
MNFPRASRLMQAAVLGGLMAVSAAATAQTNPYARGPDPTAASLEASAGPFTVRSFTVSRPSGYGAGTVYYPTNAGGTVGAIAIVPGYTARQSSIKWWGPRLASHGFVVITIDTNSTLDQPESRSSQQMAALEQVASLNGTSSSPIYGKVDTARMGVMGWSMGGGGSLISACNNPSLKAAVVQAPWHSSTNFSCVTVPTLIFCCENDSIAPCNSYALPIYDSMSENAKQFLEICGGSHSCANTGNSDQALIGKKGVAWMKRFMDNDTRYSTFACECPNSTRVCDCRTANCS